European Patent Specification EP 3 541 841 B1, published September 11, 2024. Title: ANTI-PD-1 ANTIBODIES AND COMPOSITIONS. Applicant: SYMPHOGEN A/S. Application Not yet assigned. The sequence listing filed with the application follows.

SEQUENCE LISTING (115 sequences)

SEQ ID NO: 1 - protein, 117 aa, Artificial Sequence
  source: /note="Description of Artificial Sequence: Synthetic polypeptide"
  VARIANT (35)..(35): /replace="Ser"
  VARIANT (84)..(84): /replace="Asn"
  MISC_FEATURE (1)..(117): /note="Variant residues given in the sequence have no preference with respect to those in the annotations for variant positions"
QVQLVESGGGLVKPGGSLRLSCAASGFTFSDYYMNWIRQAPGKGLEWVSYISSTGSTIYYADSVKGRFTISRDNAKNSLYLQMDSLRAEDTAVYYCARATNWGSDYWGQGTLVTVSS

SEQ ID NO: 2 - protein, 113 aa, Artificial Sequence
  source: /note="Description of Artificial Sequence: Synthetic polypeptide"
  VARIANT (1)..(1): /replace="Asp"
  VARIANT (40)..(40): /replace="Ala"
  VARIANT (55)..(55): /replace="Tyr"
  MISC_FEATURE (1)..(113): /note="Variant residues given in the sequence have no preference with respect to those in the annotations for variant positions"
EIVMTQSPDSLAVSLGERATINCKSSQSVLYSSNNKNYLFWYQQKPGQPPKLLIFWASTRESGVPDRFSGSGSGTDFTLTISSLQAEDVAVYYCQQYYSTPYTFGQGTKVEIK

SEQ ID NO: 3 - protein, 117 aa, Artificial Sequence
  source: /note="Description of Artificial Sequence: Synthetic polypeptide"
QVQLVESGGGVVQPGRSLRLSCAASGFTFSNYGMHWVRQAPGKGLEWVAVIWYDGSDKYYADSVKGRFTISRDNSKNTLYLQMNSLRAEDTAVYYCAGGGNYYGDFWGQGTLVTVSS

SEQ ID NO: 4 - protein, 107 aa, Artificial Sequence
  source: /note="Description of Artificial Sequence: Synthetic polypeptide"
  VARIANT (1)..(1): /replace="Asp"
  VARIANT (3)..(3): /replace="Gln"
  VARIANT (53)..(53): /replace="Ser"
  MISC_FEATURE (1)..(107): /note="Variant residues given in the sequence have no preference with respect to those in the annotations for variant positions"
EIVMTQSPSSLSASVGDRVTITCRASQGIRNDLGWYQQKPGKAPKRLIYVASNLQSGVPSRFSGSGSGTEFTLTISSLQPEDFATYYCLQYNSYPWTFGQGTKVEIK

SEQ ID NO: 5 - protein, 120 aa, Artificial Sequence
  source: /note="Description of Artificial Sequence: Synthetic polypeptide"
  VARIANT (1)..(1): /replace="Glu"
  VARIANT (5)..(5): /replace="Val"
  VARIANT (13)..(13): /replace="Gln"
  VARIANT (35)..(35): /replace="Ser"
  VARIANT (46)..(46): /replace="Glu"
  VARIANT (50)..(50): /replace="Ala"
  VARIANT (77)..(77): /replace="Asn"
  VARIANT (80)..(80): /replace="Tyr"
  VARIANT (115)..(115): /replace="Met"
  MISC_FEATURE (1)..(120): /note="Variant residues given in the sequence have no preference with respect to those in the annotations for variant positions"
QVQLQESGGGLVRPGGSLRLSCAASGFTFSSFAMNWVRQAPGKGLVWVSTITGGGTTSYYADSVKGRFTISRDNSKSTLFLQMNSLRAEDTAVYYCAKWGSWSAGAFDIWGQGTTVTVSS

SEQ ID NO: 6 - protein, 107 aa, Artificial Sequence
  source: /note="Description of Artificial Sequence: Synthetic polypeptide"
  VARIANT (4)..(4): /replace="Met"
  MISC_FEATURE (1)..(107): /note="Variant residues given in the sequence have no preference with respect to those in the annotations for variant positions"
DIQLTQSPSSVSASVGDRVTITCRASQGISSWLAWYQQKPGKAPKLLIYAASSLQSGVPSRFSGSGSGTDFTLTISSLQPEDFATYYCQQANSFPWTFGQGTKVEIK

SEQ ID NO: 7 - protein, 117 aa, Artificial Sequence
  source: /note="Description of Artificial Sequence: Synthetic polypeptide"
  VARIANT (64)..(64): /replace="Val"
  MISC_FEATURE (1)..(117): /note="Variant residues given in the sequence have no preference with respect to those in the annotations for variant positions"
QVQLVESGGGLVKPGGSLRLSCAASGFTFSDYYMSWIRQAPGKGLEWVSYISSSGSTIYYADSAKGRFTISRDNAKNSLYLQMNSLRAEDTAVYYCARDTNWAFDYWGQGTLVTVSS

SEQ ID NO: 8 - protein, 113 aa, Artificial Sequence
  source: /note="Description of Artificial Sequence: Synthetic polypeptide"
  VARIANT (3)..(3): /replace="Val"
  VARIANT (4)..(4): /replace="Met"
  VARIANT (69)..(69): /replace="Ser"
  MISC_FEATURE (1)..(113): /note="Variant residues given in the sequence have no preference with respect to those in the annotations for variant positions"
DIQLTQSPDSLAVSLGERATINCKSSQSVFYSANNKNYLAWYQQKPGQPPKLLIYWTSTRESGVPDRFRGSGSGTDFTLTISSLQAEDVAVYYCQQFYSTPRTFGQGTKVEIK

SEQ ID NO: 9 - protein, 119 aa, Artificial Sequence
  source: /note="Description of Artificial Sequence: Synthetic polypeptide"
  VARIANT (5)..(5): /replace="Gln"
  VARIANT (59)..(59): /replace="Asn"
  VARIANT (76)..(76): /replace="Lys"
  VARIANT (83)..(83): /replace="Leu"
  MISC_FEATURE (1)..(119): /note="Variant residues given in the sequence have no preference with respect to those in the annotations for variant positions"
QVQLVESGPGLVKPSGTLSLTCAVSGGSISSNNWWSWVRQPPGKGLEWIGEIYHDGTTTYNPSLKSRVTISVDKSRNQFSLKMSSVTAADTAVYYCARGDWGSGAFDIWGQGTMVTVSS

SEQ ID NO: 10 - protein, 107 aa, Artificial Sequence
  source: /note="Description of Artificial Sequence: Synthetic polypeptide"
  VARIANT (1)..(1): /replace="Ala"
  MISC_FEATURE (1)..(107): /note="Variant residues given in the sequence have no preference with respect to those in the annotations for variant positions"
DIQMTQSPSSLSASVGDRVTITCRASQGIRNDLGWYQQKPGKAPKLLIYAASSLQSGVPSRFSGSGSGTDFTLTISSLQPEDFATYYCLQDYNYPRTFGQGTKVEIK

SEQ ID NO: 11 - protein, 117 aa, Artificial Sequence
  source: /note="Description of Artificial Sequence: Synthetic polypeptide"
  VARIANT (10)..(10): /replace="Gly"
  VARIANT (16)..(16): /replace="Gly"
  MISC_FEATURE (1)..(117): /note="Variant residues given in the sequence have no preference with respect to those in the annotations for variant positions"
QVQLVESGGDLVKPGRSLRLSCAASGFTFSDYYMSWIRQAPGKGLEWVSYISSSSSTIYYADSVKGRFTISRDNAKNSLYLQMNSLRAEDTAVYYCARDTNWAFDYWGQGTLVTVSS

SEQ ID NO: 12 - protein, 113 aa, Artificial Sequence
  source: /note="Description of Artificial Sequence: Synthetic polypeptide"
  VARIANT (1)..(1): /replace="Asp"
  VARIANT (4)..(4): /replace="Met"
  VARIANT (55)..(55): /replace="Tyr"
  VARIANT (93)..(93): /replace="Tyr"
  MISC_FEATURE (1)..(113): /note="Variant residues given in the sequence have no preference with respect to those in the annotations for variant positions"
EIVLTQSPDSLAVSLGERATINCKSSQSVFYSSNNKNYLAWYQQKPGQPPKLLIFWASTRESGVPDRFSGSGSGTDFTLTISSLQAEDVAVYFCQQFYSTPRTFGQGTKVEIK

SEQ ID NO: 13 - protein, 117 aa, Artificial Sequence
  source: /note="Description of Artificial Sequence: Synthetic polypeptide"
  VARIANT (5)..(5): /replace="Val"
  VARIANT (50)..(50): /replace="Tyr"
  VARIANT (59)..(59): /replace="Tyr"
  VARIANT (61)..(61): /replace="Ala"
  MISC_FEATURE (1)..(117): /note="Variant residues given in the sequence have no preference with respect to those in the annotations for variant positions"
QVQLQESGGGLVKPGGSLRLSCAASGFTFRDYYMSWIRQAPGKGLEWVSHISSSGSIIDYVDSVKGRFTISRDNAKNSLYLQMNSLRAEDTAVYYCARDTNWALDYWGQGTLVTVSS

SEQ ID NO: 14 - protein, 113 aa, Artificial Sequence
  source: /note="Description of Artificial Sequence: Synthetic polypeptide"
  VARIANT (3)..(3): /replace="Val"
  VARIANT (4)..(4): /replace="Met"
  VARIANT (55)..(55): /replace="Tyr"
  MISC_FEATURE (1)..(113): /note="Variant residues given in the sequence have no preference with respect to those in the annotations for variant positions"
DIQLTQSPDSLAVSLGERATINCKSSQSVFYSSNNKNYLAWYQQKPGQPPKLLISWASTRESGVPDRFSGSGSGTDFTLTISSLQAEDVAVYYCQQYYSTPYTFGQGTKLEIK

SEQ ID NO: 15 - protein, 120 aa, Artificial Sequence
  source: /note="Description of Artificial Sequence: Synthetic polypeptide"
  VARIANT (1)..(1): /replace="Glu"
  VARIANT (5)..(5): /replace="Val"
  VARIANT (6)..(6): /replace="Glu"
  VARIANT (35)..(35): /replace="Ser"
  VARIANT (49)..(49): /replace="Ser"
  VARIANT (50)..(50): /replace="Ala"
  VARIANT (73)..(73): /replace="Asp"
  VARIANT (78)..(78): /replace="Thr"
  MISC_FEATURE (1)..(120): /note="Variant residues given in the sequence have no preference with respect to those in the annotations for variant positions"
QVQLQQSGGGLVQPGGSLRLSCAASGFTFSSHVMNWVRQAPGKGLEWVATISGSGVDTYYADSVKGRFTISRGNSKNMLYLQMNSLRAEDTAVYYCAKWGSWSAGAFDIWGQGTMVTVSS

SEQ ID NO: 16 - protein, 107 aa, Artificial Sequence
  source: /note="Description of Artificial Sequence: Synthetic polypeptide"
  VARIANT (1)..(1): /replace="Asp"
  VARIANT (3)..(3): /replace="Gln"
  VARIANT (4)..(4): /replace="Met"
  MISC_FEATURE (1)..(107): /note="Variant residues given in the sequence have no preference with respect to those in the annotations for variant positions"
EIVLTQSPSSVSASVGDRVTITCRASQGISSWLAWYQQKPGKAPKLLIYAASSLQSGVPSRFSGSGSGTDFTLTISSLQPEDFATYYCQQANSFPWTFGQGTKVEIK

SEQ ID NO: 17 - protein, 117 aa, Artificial Sequence
  source: /note="Description of Artificial Sequence: Synthetic polypeptide"
  VARIANT (1)..(1): /replace="Glu"
  VARIANT (6)..(6): /replace="Glu"
  MISC_FEATURE (1)..(117): /note="Variant residues given in the sequence have no preference with respect to those in the annotations for variant positions"
QVQLVQSGGGLVQPGGSLRLSCAASGFTFSSYWMSWVRQAPGKGLEWVANIKQDGSEKYYVDSVKGRFTISRDNAKNSLYLQMNSLRAEDTAVYYCARDTNWGFDNWGQGTLVTVSS

SEQ ID NO: 18 - protein, 113 aa, Artificial Sequence
  source: /note="Description of Artificial Sequence: Synthetic polypeptide"
  VARIANT (1)..(1): /replace="Asp"
  VARIANT (40)..(40): /replace="Ala"
  VARIANT (55)..(55): /replace="Tyr"
  MISC_FEATURE (1)..(113): /note="Variant residues given in the sequence have no preference with respect to those in the annotations for variant positions"
EIVMTQSPDSLAVSLGERATINCKSSQSVLYSSNNKNYLLWYQQKPGQPPKLLIFWASTRESGVPDRFSGSGSGTDFTLTISSLQAEDVAVYYCQQYYSTPYTFGQGTKLEIK

SEQ ID NO: 19 - protein, 119 aa, Artificial Sequence
  source: /note="Description of Artificial Sequence: Synthetic polypeptide"
  VARIANT (2)..(2): /replace="Val"
  VARIANT (43)..(43): /replace="Gly"
  VARIANT (49)..(49): /replace="Ile"
  VARIANT (59)..(59): /replace="Asn"
  VARIANT (70)..(70): /replace="Ile"
  VARIANT (111)..(111): /replace="Gln"
  MISC_FEATURE (1)..(119): /note="Variant residues given in the sequence have no preference with respect to those in the annotations for variant positions"
QLQLQESGPGLVKPSGTLSLTCAVSGGSISSSNWWSWVRQPPKKGLEWVGEIFHDGTTSYNPSLKSRVTMSVDKSKNQFSLKLSSVTAADTAVYYCARGNWGSGALDIWGPGTMVTVSS

SEQ ID NO: 20 - protein, 107 aa, Artificial Sequence
  source: /note="Description of Artificial Sequence: Synthetic polypeptide"
  VARIANT (1)..(1): /replace="Ala"
  VARIANT (3)..(3): /replace="Gln"
  VARIANT (10)..(10): /replace="Ser"
  MISC_FEATURE (1)..(107): /note="Variant residues given in the sequence have no preference with respect to those in the annotations for variant positions"
EIVMTQSPSPLSASVGDRVTITCRASQGIRNDLGWYQQKPGKAPKLLIYAASSLQSGVPSRFSGSGSGTDFTLTISSLQPEDFATYYCLQDYNYPRTFGQGTKVEIK

SEQ ID NO: 21 - protein, 118 aa, Artificial Sequence
  source: /note="Description of Artificial Sequence: Synthetic polypeptide"
  VARIANT (48)..(48): /replace="Val"
  VARIANT (50)..(50): /replace="Ala"
  MISC_FEATURE (1)..(118): /note="Variant residues given in the sequence have no preference with respect to those in the annotations for variant positions"
EVQLVESGGGLVQPGGSLRLSCAASGFTFSSFVMSWVRQAPGKGLEWLSTISGGGGSTYYADSVKGRFTISRDNSKNTLYLQMNSLRAEDTAVYYCAKDWDLYYFDYWGQGTLVTVSS

SEQ ID NO: 22 - protein, 107 aa, Artificial Sequence
  source: /note="Description of Artificial Sequence: Synthetic polypeptide"
  VARIANT (4)..(4): /replace="Met"
  VARIANT (12)..(12): /replace="Ser"
  MISC_FEATURE (1)..(107): /note="Variant residues given in the sequence have no preference with respect to those in the annotations for variant positions"
DIQLTQSPSSVPASVGDRVTITCRASQGISNWLAWYQQKPGKAPKLLIYAASSLQSGVPSRFSGSGSGTDFTLTISSLQPEDFATYYCQQANSFPLTFGGGTKVEIK

SEQ ID NO: 23 - protein, 117 aa, Artificial Sequence
  source: /note="Description of Artificial Sequence: Synthetic polypeptide"
  VARIANT (1)..(1): /replace="Glu"
  VARIANT (5)..(5): /replace="Val"
  VARIANT (6)..(6): /replace="Glu"
  VARIANT (35)..(35): /replace="Ser"
  MISC_FEATURE (1)..(117): /note="Variant residues given in the sequence have no preference with respect to those in the annotations for variant positions"
QVQLQQSGGGLVQPGGSLRLSCAASGFTFSDYWMNWVRQAPGKGLEWVANIKEDGNEKYYVDSVKGRFTISRDNAKNSLYLQMNSLRAEDTAVYYCARDTNWGSDYWGQGTLVTVSS

SEQ ID NO: 24 - protein, 113 aa, Artificial Sequence
  source: /note="Description of Artificial Sequence: Synthetic polypeptide"
  VARIANT (3)..(3): /replace="Val"
  VARIANT (40)..(40): /replace="Ala"
  VARIANT (55)..(55): /replace="Tyr"
  MISC_FEATURE (1)..(113): /note="Variant residues given in the sequence have no preference with respect to those in the annotations for variant positions"
DIQMTQSPDSLAVSLGERATINCKSSQSVFYSSNNKNYLLWYQQKPGQPPKLLIFWASTRESGVPDRFSGSGSGTDFTLTISSLQAEDVAVYYCQQYYSTPYTFGQGTKLEIK

SEQ ID NO: 25 - DNA, 990 bp, Artificial Sequence
  source: /note="Description of Artificial Sequence: Synthetic polynucleotide"
gcctccaccaagggcccatcggtcttccccctggcaccctcctccaagagcacctctgggggcacagcggccctgggctgcctggtcaaggactacttccccgaaccggtgacggtgtcgtggaactcaggcgccctgaccagcggcgtgcacaccttcccggctgtcctacagtcctcaggactctactccctcagcagcgtggtgaccgtgccctccagcagcttgggcacccagacctacatctgcaacgtgaatcacaagcccagcaacaccaaggtggacaagagagttgagcccaaatcttgtgacaaaactcacacatgcccaccgtgcccagcacctgaagccgccgggggaccgtcagtcttcctcttccccccaaaacccaaggacaccctcatgatctcccggacccctgaggtcacatgcgtggtggtggacgtgagccacgaagaccctgaggtcaagttcaactggtacgtggacggcgtggaggtgcataatgccaagacaaagccgcgggaggagcagtacaacagcacgtaccgtgtggtcagcgtcctcaccgtcctgcaccaggactggctgaatggcaaggagtacaagtgcaaggtctccaacaaagccctcccagcccccatcgagaaaaccatctccaaagccaaagggcagccccgagaaccacaggtgtacaccctgcccccatcccgggaggagatgaccaagaaccaggtcagcctgacctgcctggtcaaaggcttctatcccagcgacatcgccgtggagtgggagagcaatgggcagccggagaacaactacaagaccacgcctcccgtgctggactccgacggctccttcttcctctatagcaagctcaccgtggacaagagcaggtggcagcaggggaacgtcttctcatgctccgtgatgcatgaggctctgcacaaccactacacgcagaagagcctctccctgtccccgggtaaa

SEQ ID NO: 26 - protein, 330 aa, Artificial Sequence
  source: /note="Description of Artificial Sequence: Synthetic polypeptide"
ASTKGPSVFPLAPSSKSTSGGTAALGCLVKDYFPEPVTVSWNSGALTSGVHTFPAVLQSSGLYSLSSVVTVPSSSLGTQTYICNVNHKPSNTKVDKRVEPKSCDKTHTCPPCPAPEAAGGPSVFLFPPKPKDTLMISRTPEVTCVVVDVSHEDPEVKFNWYVDGVEVHNAKTKPREEQYNSTYRVVSVLTVLHQDWLNGKEYKCKVSNKALPAPIEKTISKAKGQPREPQVYTLPPSREEMTKNQVSLTCLVKGFYPSDIAVEWESNGQPENNYKTTPPVLDSDGSFFLYSKLTVDKSRWQQGNVFSCSVMHEALHNHYTQKSLSLSPGK

SEQ ID NO: 27 - DNA, 321 bp, Artificial Sequence
  source: /note="Description of Artificial Sequence: Synthetic polynucleotide"
cgtacggtggctgcaccatctgtcttcatcttcccgccatctgatgagcagttgaaatctggaactgcctctgttgtgtgcctgctgaataacttctatcccagagaggccaaagtacagtggaaggtggataacgccctccaatcgggtaactcccaggagagtgtcacagagcaggacagcaaggacagcacctacagcctcagcagcaccctgacgctgagcaaagcagactacgagaaacacaaagtctacgcctgcgaagtcacccatcagggcctgagctcgcccgtcacaaagagcttcaacaggggagagtgt

SEQ ID NO: 28 - protein, 107 aa, Artificial Sequence [sequence omitted]

SEQ ID NO: 29 - protein, 8 aa, Artificial Sequence
  source: /note="Description of Artificial Sequence: Synthetic peptide"
GFTFSDYY

SEQ ID NO: 30 - protein, 8 aa, Artificial Sequence
  source: /note="Description of Artificial Sequence: Synthetic peptide"
ISSTGSTI

SEQ ID NO: 31 - protein, 11 aa, Artificial Sequence
  source: /note="Description of Artificial Sequence: Synthetic peptide"
CARATNWGSDY

SEQ ID NO: 32 - protein, 12 aa, Artificial Sequence
  source: /note="Description of Artificial Sequence: Synthetic peptide"
QSVLYSSNNKNY

SEQ ID NO: 33 - protein, 3 aa, Artificial Sequence
  source: /note="Description of Artificial Sequence: Synthetic peptide"
WAS

SEQ ID NO: 34 - protein, 10 aa, Artificial Sequence
  source: /note="Description of Artificial Sequence: Synthetic peptide"
CQQYYSTPYT

SEQ ID NO: 35 - protein, 8 aa, Artificial Sequence
  source: /note="Description of Artificial Sequence: Synthetic peptide"
GFTFSNYG

SEQ ID NO: 36 - protein, 8 aa, Artificial Sequence
  source: /note="Description of Artificial Sequence: Synthetic peptide"
IWYDGSDK

SEQ ID NO: 37 - protein, 11 aa, Artificial Sequence
  source: /note="Description of Artificial Sequence: Synthetic peptide"
CAGGGNYYGDF

SEQ ID NO: 38 - protein, 6 aa, Artificial Sequence
  source: /note="Description of Artificial Sequence: Synthetic peptide"
QGIRND

SEQ ID NO: 39 - protein, 3 aa, Artificial Sequence
  source: /note="Description of Artificial Sequence: Synthetic peptide"
VAS

SEQ ID NO: 40 - protein, 10 aa, Artificial Sequence
  source: /note="Description of Artificial Sequence: Synthetic peptide"
CLQYNSYPWT

SEQ ID NO: 41 - protein, 8 aa, Artificial Sequence
  source: /note="Description of Artificial Sequence: Synthetic peptide"
GFTFSSFA

SEQ ID NO: 42 - protein, 8 aa, Artificial Sequence
  source: /note="Description of Artificial Sequence: Synthetic peptide"
ITGGGTTS

SEQ ID NO: 43 - protein, 14 aa, Artificial Sequence
  source: /note="Description of Artificial Sequence: Synthetic peptide"
CAKWGSWSAGAFDI

SEQ ID NO: 44 - protein, 6 aa, Artificial Sequence
  source: /note="Description of Artificial Sequence: Synthetic peptide"
QGISSW

SEQ ID NO: 45 - protein, 3 aa, Artificial Sequence
  source: /note="Description of Artificial Sequence: Synthetic peptide"
AAS

SEQ ID NO: 46 - protein, 10 aa, Artificial Sequence
  source: /note="Description of Artificial Sequence: Synthetic peptide"
CQQANSFPWT

SEQ ID NO: 47 - protein, 8 aa, Artificial Sequence
  source: /note="Description of Artificial Sequence: Synthetic peptide"
ISSSGSTI

SEQ ID NO: 48 - protein, 11 aa, Artificial Sequence
  source: /note="Description of Artificial Sequence: Synthetic peptide"
CARDTNWAFDY

SEQ ID NO: 49 - protein, 12 aa, Artificial Sequence
  source: /note="Description of Artificial Sequence: Synthetic peptide"
QSVFYSANNKNY

SEQ ID NO: 50 - protein, 3 aa, Artificial Sequence
  source: /note="Description of Artificial Sequence: Synthetic peptide"
WTS

SEQ ID NO: 51 - protein, 10 aa, Artificial Sequence
  source: /note="Description of Artificial Sequence: Synthetic peptide"
CQQFYSTPRT

SEQ ID NO: 52 - protein, 9 aa, Artificial Sequence
  source: /note="Description of Artificial Sequence: Synthetic peptide"
GGSISSNNW

SEQ ID NO: 53 - protein, 7 aa, Artificial Sequence
  source: /note="Description of Artificial Sequence: Synthetic peptide"
IYHDGTT

SEQ ID NO: 54 - protein, 13 aa, Artificial Sequence
  source: /note="Description of Artificial Sequence: Synthetic peptide"
CARGDWGSGAFDI

SEQ ID NO: 55 - protein, 10 aa, Artificial Sequence
  source: /note="Description of Artificial Sequence: Synthetic peptide"
CLQDYNYPRT

SEQ ID NO: 56 - protein, 8 aa, Artificial Sequence
  source: /note="Description of Artificial Sequence: Synthetic peptide"
ISSSSSTI

SEQ ID NO: 57 - protein, 12 aa, Artificial Sequence
  source: /note="Description of Artificial Sequence: Synthetic peptide"
QSVFYSSNNKNY

SEQ ID NO: 58 - protein, 8 aa, Artificial Sequence
  source: /note="Description of Artificial Sequence: Synthetic peptide"
GFTFRDYY

SEQ ID NO: 59 - protein, 8 aa, Artificial Sequence
  source: /note="Description of Artificial Sequence: Synthetic peptide"
ISSSGSII

SEQ ID NO: 60 - protein, 11 aa, Artificial Sequence
  source: /note="Description of Artificial Sequence: Synthetic peptide"
CARDTNWALDY

SEQ ID NO: 61 - protein, 8 aa, Artificial Sequence
  source: /note="Description of Artificial Sequence: Synthetic peptide"
GFTFSSHV

SEQ ID NO: 62 - protein, 8 aa, Artificial Sequence
  source: /note="Description of Artificial Sequence: Synthetic peptide"
ISGSGVDT

SEQ ID NO: 63 - protein, 8 aa, Artificial Sequence
  source: /note="Description of Artificial Sequence: Synthetic peptide"
GFTFSSYW

SEQ ID NO: 64 - protein, 8 aa, Artificial Sequence
  source: /note="Description of Artificial Sequence: Synthetic peptide"
IKQDGSEK

SEQ ID NO: 65 - protein, 11 aa, Artificial Sequence
  source: /note="Description of Artificial Sequence: Synthetic peptide"
CARDTNWGFDN

SEQ ID NO: 66 - protein, 9 aa, Artificial Sequence
  source: /note="Description of Artificial Sequence: Synthetic peptide"
GGSISSSNW

SEQ ID NO: 67 - protein, 7 aa, Artificial Sequence
  source: /note="Description of Artificial Sequence: Synthetic peptide"
IFHDGTT

SEQ ID NO: 68 - protein, 13 aa, Artificial Sequence
  source: /note="Description of Artificial Sequence: Synthetic peptide"
CARGNWGSGALDI

SEQ ID NO: 69 - protein, 8 aa, Artificial Sequence
  source: /note="Description of Artificial Sequence: Synthetic peptide"
GFTFSSFV

SEQ ID NO: 70 - protein, 8 aa, Artificial Sequence
  source: /note="Description of Artificial Sequence: Synthetic peptide"
ISGGGGST

SEQ ID NO: 71 - protein, 12 aa, Artificial Sequence
  source: /note="Description of Artificial Sequence: Synthetic peptide"
CAKDWDLYYFDY

SEQ ID NO: 72 - protein, 6 aa, Artificial Sequence
  source: /note="Description of Artificial Sequence: Synthetic peptide"
QGISNW

SEQ ID NO: 73 - protein, 10 aa, Artificial Sequence
  source: /note="Description of Artificial Sequence: Synthetic peptide"
CQQANSFPLT

SEQ ID NO: 74 - protein, 8 aa, Artificial Sequence
  source: /note="Description of Artificial Sequence: Synthetic peptide"
GFTFSDYW

SEQ ID NO: 75 - protein, 8 aa, Artificial Sequence
  source: /note="Description of Artificial Sequence: Synthetic peptide"
IKEDGNEK

SEQ ID NO: 76 - protein, 11 aa, Artificial Sequence
  source: /note="Description of Artificial Sequence: Synthetic peptide"
CARDTNWGSDY

SEQ ID NO: 77 - protein, 120 aa, Artificial Sequence
  source: /note="Description of Artificial Sequence: Synthetic polypeptide"
EVQLVESGGGLVQPGGSLRLSCAASGFTFSSFAMSWVRQAPGKGLVWVSTITGGGTTSYYADSVKGRFTISRDNSKSTLFLQMNSLRAEDTAVYYCAKWGSWSAGAFDIWGQGTTVTVSS

SEQ ID NO: 78 - protein, 119 aa, Artificial Sequence
  source: /note="Description of Artificial Sequence: Synthetic polypeptide"
QVQLQESGPGLVKPSGTLSLTCAVSGGSISSNNWWSWVRQPPGKGLEWIGEIYHDGTTTYNPSLKSRVTISVDKSRNQFSLKMSSVTAADTAVYYCARGDWGSGAFDIWGQGTMVTVSS

SEQ ID NO: 79 - protein, 117 aa, Artificial Sequence
  source: /note="Description of Artificial Sequence: Synthetic polypeptide"
QVQLVESGGGLVKPGGSLRLSCAASGFTFRDYYMSWIRQAPGKGLEWVSHISSSGSIIDYVDSVKGRFTISRDNAKNSLYLQMNSLRAEDTAVYYCARDTNWALDYWGQGTLVTVSS

SEQ ID NO: 80 - protein, 120 aa, Artificial Sequence
  source: /note="Description of Artificial Sequence: Synthetic polypeptide"
EVQLVESGGGLVQPGGSLRLSCAASGFTFSSHVMNWVRQAPGKGLEWVATISGSGVDTYYADSVKGRFTISRGNSKNMLYLQMNSLRAEDTAVYYCAKWGSWSAGAFDIWGQGTMVTVSS

SEQ ID NO: 81 - protein, 117 aa, Artificial Sequence
  source: /note="Description of Artificial Sequence: Synthetic polypeptide"
EVQLVESGGGLVQPGGSLRLSCAASGFTFSSYWMSWVRQAPGKGLEWVANIKQDGSEKYYVDSVKGRFTISRDNAKNSLYLQMNSLRAEDTAVYYCARDTNWGFDNWGQGTLVTVSS

SEQ ID NO: 82 - protein, 119 aa, Artificial Sequence
  source: /note="Description of Artificial Sequence: Synthetic polypeptide"
QVQLQESGPGLVKPSGTLSLTCAVSGGSISSSNWWSWVRQPPKKGLEWVGEIFHDGTTSYNPSLKSRVTMSVDKSKNQFSLKLSSVTAADTAVYYCARGNWGSGALDIWGPGTMVTVSS

SEQ ID NO: 83 - protein, 117 aa, Artificial Sequence
  source: /note="Description of Artificial Sequence: Synthetic polypeptide"
EVQLVESGGGLVQPGGSLRLSCAASGFTFSDYWMNWVRQAPGKGLEWVANIKEDGNEKYYVDSVKGRFTISRDNAKNSLYLQMNSLRAEDTAVYYCARDTNWGSDYWGQGTLVTVSS

SEQ ID NO: 84 - protein, 113 aa, Artificial Sequence
  source: /note="Description of Artificial Sequence: Synthetic polypeptide"
DIVMTQSPDSLAVSLGERATINCKSSQSVLYSSNNKNYLFWYQQKPGQPPKLLIFWASTRESGVPDRFSGSGSGTDFTLTISSLQAEDVAVYYCQQYYSTPYTFGQGTKVEIK

SEQ ID NO: 85 - protein, 107 aa, Artificial Sequence
  source: /note="Description of Artificial Sequence: Synthetic polypeptide"
DIQMTQSPSSLSASVGDRVTITCRASQGIRNDLGWYQQKPGKAPKRLIYVASNLQSGVPSRFSGSGSGTEFTLTISSLQPEDFATYYCLQYNSYPWTFGQGTKVEIK

SEQ ID NO: 86 - protein, 107 aa, Artificial Sequence; identical to SEQ ID NO: 6
  source: /note="Description of Artificial Sequence: Synthetic polypeptide"

SEQ ID NO: 87 - protein, 113 aa, Artificial Sequence
  source: /note="Description of Artificial Sequence: Synthetic polypeptide"
DIVMTQSPDSLAVSLGERATINCKSSQSVFYSANNKNYLAWYQQKPGQPPKLLIYWTSTRESGVPDRFRGSGSGTDFTLTISSLQAEDVAVYYCQQFYSTPRTFGQGTKVEIK

SEQ ID NO: 88 - protein, 107 aa, Artificial Sequence
  source: /note="Description of Artificial Sequence: Synthetic polypeptide"
AIQMTQSPSSLSASVGDRVTITCRASQGIRNDLGWYQQKPGKAPKLLIYAASSLQSGVPSRFSGSGSGTDFTLTISSLQPEDFATYYCLQDYNYPRTFGQGTKVEIK

SEQ ID NO: 89 - protein, 113 aa, Artificial Sequence
  source: /note="Description of Artificial Sequence: Synthetic polypeptide"
DIVMTQSPDSLAVSLGERATINCKSSQSVFYSSNNKNYLAWYQQKPGQPPKLLIFWASTRESGVPDRFSGSGSGTDFTLTISSLQAEDVAVYFCQQFYSTPRTFGQGTKVEIK

SEQ ID NO: 90 - protein, 113 aa, Artificial Sequence
  source: /note="Description of Artificial Sequence: Synthetic polypeptide"
DIVMTQSPDSLAVSLGERATINCKSSQSVFYSSNNKNYLAWYQQKPGQPPKLLISWASTRESGVPDRFSGSGSGTDFTLTISSLQAEDVAVYYCQQYYSTPYTFGQGTKLEIK

SEQ ID NO: 91 - protein, 107 aa, Artificial Sequence
  source: /note="Description of Artificial Sequence: Synthetic polypeptide"
DIQMTQSPSSVSASVGDRVTITCRASQGISSWLAWYQQKPGKAPKLLIYAASSLQSGVPSRFSGSGSGTDFTLTISSLQPEDFATYYCQQANSFPWTFGQGTKVEIK

SEQ ID NO: 92 - protein, 113 aa, Artificial Sequence
  source: /note="Description of Artificial Sequence: Synthetic polypeptide"
DIVMTQSPDSLAVSLGERATINCKSSQSVLYSSNNKNYLLWYQQKPGQPPKLLIFWASTRESGVPDRFSGSGSGTDFTLTISSLQAEDVAVYYCQQYYSTPYTFGQGTKLEIK

SEQ ID NO: 93 - protein, 107 aa, Artificial Sequence
  source: /note="Description of Artificial Sequence: Synthetic polypeptide"
AIQMTQSPSPLSASVGDRVTITCRASQGIRNDLGWYQQKPGKAPKLLIYAASSLQSGVPSRFSGSGSGTDFTLTISSLQPEDFATYYCLQDYNYPRTFGQGTKVEIK

SEQ ID NO: 94 - protein, 107 aa, Artificial Sequence; identical to SEQ ID NO: 22
  source: /note="Description of Artificial Sequence: Synthetic polypeptide"

SEQ ID NO: 95 - protein, 113 aa, Artificial Sequence
  source: /note="Description of Artificial Sequence: Synthetic polypeptide"
DIVMTQSPDSLAVSLGERATINCKSSQSVFYSSNNKNYLLWYQQKPGQPPKLLIFWASTRESGVPDRFSGSGSGTDFTLTISSLQAEDVAVYYCQQYYSTPYTFGQGTKLEIK

SEQ ID NO: 96 - protein, 117 aa, Artificial Sequence
  source: /note="Description of Artificial Sequence: Synthetic polypeptide"
QVQLVESGGGLVKPGGSLRLSCAASGFTFSDYYMSWIRQAPGKGLEWVSYISSTGSTIYYADSVKGRFTISRDNAKNSLYLQMNSLRAEDTAVYYCARATNWGSDYWGQGTLVTVSS

SEQ ID NO: 97 - protein, 120 aa, Artificial Sequence
  source: /note="Description of Artificial Sequence: Synthetic polypeptide"
EVQLVESGGGLVQPGGSLRLSCAASGFTFSSFAMSWVRQAPGKGLEWVSAITGGGTTSYYADSVKGRFTISRDNSKNTLYLQMNSLRAEDTAVYYCAKWGSWSAGAFDIWGQGTMVTVSS

SEQ ID NO: 98 - protein, 117 aa, Artificial Sequence
  source: /note="Description of Artificial Sequence: Synthetic polypeptide"
QVQLVESGGGLVKPGGSLRLSCAASGFTFSDYYMSWIRQAPGKGLEWVSYISSSGSTIYYADSVKGRFTISRDNAKNSLYLQMNSLRAEDTAVYYCARDTNWAFDYWGQGTLVTVSS

SEQ ID NO: 99 - protein, 119 aa, Artificial Sequence
  source: /note="Description of Artificial Sequence: Synthetic polypeptide"
QVQLQESGPGLVKPSGTLSLTCAVSGGSISSNNWWSWVRQPPGKGLEWIGEIYHDGTTNYNPSLKSRVTISVDKSKNQFSLKLSSVTAADTAVYYCARGDWGSGAFDIWGQGTMVTVSS

SEQ ID NO: 100 - protein, 117 aa, Artificial Sequence
  source: /note="Description of Artificial Sequence: Synthetic polypeptide"
QVQLVESGGGLVKPGGSLRLSCAASGFTFSDYYMSWIRQAPGKGLEWVSYISSSSSTIYYADSVKGRFTISRDNAKNSLYLQMNSLRAEDTAVYYCARDTNWAFDYWGQGTLVTVSS

SEQ ID NO: 101 - protein, 117 aa, Artificial Sequence
  source: /note="Description of Artificial Sequence: Synthetic polypeptide"
QVQLVESGGGLVKPGGSLRLSCAASGFTFRDYYMSWIRQAPGKGLEWVSYISSSGSIIYYADSVKGRFTISRDNAKNSLYLQMNSLRAEDTAVYYCARDTNWALDYWGQGTLVTVSS

SEQ ID NO: 102 - protein, 120 aa, Artificial Sequence
  source: /note="Description of Artificial Sequence: Synthetic polypeptide"
EVQLVESGGGLVQPGGSLRLSCAASGFTFSSHVMNWVRQAPGKGLEWVSAISGSGVDTYYADSVKGRFTISRDNSKNTLYLQMNSLRAEDTAVYYCAKWGSWSAGAFDIWGQGTMVTVSS

SEQ ID NO: 103 - protein, 119 aa, Artificial Sequence
  source: /note="Description of Artificial Sequence: Synthetic polypeptide"
QVQLQESGPGLVKPSGTLSLTCAVSGGSISSSNWWSWVRQPPGKGLEWIGEIFHDGTTNYNPSLKSRVTISVDKSKNQFSLKLSSVTAADTAVYYCARGNWGSGALDIWGQGTMVTVSS

SEQ ID NO: 104 - protein, 118 aa, Artificial Sequence
  source: /note="Description of Artificial Sequence: Synthetic polypeptide"
EVQLVESGGGLVQPGGSLRLSCAASGFTFSSFVMSWVRQAPGKGLEWVSAISGGGGSTYYADSVKGRFTISRDNSKNTLYLQMNSLRAEDTAVYYCAKDWDLYYFDYWGQGTLVTVSS

SEQ ID NO: 105 - protein, 117 aa, Artificial Sequence
  source: /note="Description of Artificial Sequence: Synthetic polypeptide"
EVQLVESGGGLVQPGGSLRLSCAASGFTFSDYWMSWVRQAPGKGLEWVANIKEDGNEKYYVDSVKGRFTISRDNAKNSLYLQMNSLRAEDTAVYYCARDTNWGSDYWGQGTLVTVSS

SEQ ID NO: 106 - protein, 113 aa, Artificial Sequence
  source: /note="Description of Artificial Sequence: Synthetic polypeptide"
DIVMTQSPDSLAVSLGERATINCKSSQSVLYSSNNKNYLAWYQQKPGQPPKLLIYWASTRESGVPDRFSGSGSGTDFTLTISSLQAEDVAVYYCQQYYSTPYTFGQGTKVEIK

SEQ ID NO: 107 - protein, 107 aa, Artificial Sequence
  source: /note="Description of Artificial Sequence: Synthetic polypeptide"
DIQMTQSPSSLSASVGDRVTITCRASQGIRNDLGWYQQKPGKAPKRLIYVASSLQSGVPSRFSGSGSGTEFTLTISSLQPEDFATYYCLQYNSYPWTFGQGTKVEIK

SEQ ID NO: 108 - protein, 113 aa, Artificial Sequence
  source: /note="Description of Artificial Sequence: Synthetic polypeptide"
DIVMTQSPDSLAVSLGERATINCKSSQSVFYSANNKNYLAWYQQKPGQPPKLLIYWTSTRESGVPDRFSGSGSGTDFTLTISSLQAEDVAVYYCQQFYSTPRTFGQGTKVEIK

SEQ ID NO: 109 - protein, 113 aa, Artificial Sequence
  source: /note="Description of Artificial Sequence: Synthetic polypeptide"
DIVMTQSPDSLAVSLGERATINCKSSQSVFYSSNNKNYLAWYQQKPGQPPKLLIYWASTRESGVPDRFSGSGSGTDFTLTISSLQAEDVAVYYCQQFYSTPRTFGQGTKVEIK

SEQ ID NO: 110 - protein, 113 aa, Artificial Sequence
  source: /note="Description of Artificial Sequence: Synthetic polypeptide"
DIVMTQSPDSLAVSLGERATINCKSSQSVFYSSNNKNYLAWYQQKPGQPPKLLIYWASTRESGVPDRFSGSGSGTDFTLTISSLQAEDVAVYYCQQYYSTPYTFGQGTKLEIK

SEQ ID NO: 111 - protein, 113 aa, Artificial Sequence
  source: /note="Description of Artificial Sequence: Synthetic polypeptide"
DIVMTQSPDSLAVSLGERATINCKSSQSVLYSSNNKNYLAWYQQKPGQPPKLLIYWASTRESGVPDRFSGSGSGTDFTLTISSLQAEDVAVYYCQQYYSTPYTFGQGTKLEIK

SEQ ID NO: 112 - protein, 107 aa, Artificial Sequence; identical to SEQ ID NO: 88
  source: /note="Description of Artificial Sequence: Synthetic polypeptide"

SEQ ID NO: 113 - protein, 107 aa, Artificial Sequence; identical to SEQ ID NO: 22
  source: /note="Description of Artificial Sequence: Synthetic polypeptide"

SEQ ID NO: 114 - protein, 113 aa, Artificial Sequence; identical to SEQ ID NO: 110
  source: /note="Description of Artificial Sequence: Synthetic polypeptide"

SEQ ID NO: 115 - protein, 15 aa, Artificial Sequence
  source: /note="Description of Artificial Sequence: Synthetic peptide"
GGGGSGGGGSGGGGS